European Patent Application EP 4 534 665 A1, published April 9, 2025. Title: COMPOSITION FOR ENHANCING EFFICACY OF GENOME EDITING AND USE THEREOF. Applicant: 国立研究開発法人産業技術総合研究所. Application WO. The sequence listing filed with the application follows.

SEQUENCE LISTING (26 sequences)

SEQ ID NO: 1 - DNA, 309 bp, Escherichia coli
  source 1..309: mol_type = genomic DNA
  CDS 1..309
atggctaaggggcaatctttacaagatccgttcctgaacgcactgcgtcgggaacgtgttccagtttctatttatttggtgaatggtattaagctgcaagggcaaatcgagtcttttgatcagttcgtgatcctgttgaaaaacacggtcagccagatggtttacaagcacgcgatttctactgttgtcccgtctcgcccggtttctcatcacagtaacaacgccggtggcggtaccagcagtaactaccatcatggtagcagcgcgcagaatacttccgcgcaacaggacagcgaagaaaccgaataa

SEQ ID NO: 2 - protein, 102 aa, Escherichia coli
MAKGQSLQDPFLNALRRERVPVSIYLVNGIKLQGQIESFDQFVILLKNTVSQMVYKHAISTVVPSRPVSHHSNNAGGGTSSNYHHGSSAQNTSAQQDSEETE

SEQ ID NO: 3 - DNA, 249 bp, Pseudomonas aeruginosa
  source 1..249: mol_type = genomic DNA
  CDS 1..249
atgtcaaaagggcattcgctacaagacccttacctcaataccctgcggaaagaacgcgtcccggtttccatctatctggtcaacggcatcaagctgcaaggccagatcgagtctttcgaccagtttgtcatcctgctgaagaacaccgtcagccagatggtttacaagcacgcgatctccaccgtggtaccgagccgtccggtgcgtctgccgagcggtgaccagccggccgagccgggcaacgcttga

SEQ ID NO: 4 - protein, 82 aa, Pseudomonas aeruginosa
MSKGHSLQDPYLNTLRKERVPVSIYLVNGIKLQGQIESFDQFVILLKNTVSQMVYKHAISTVVPSRPVRLPSGDQPAEPGNA

SEQ ID NO: 5 - DNA, 1917 bp, Escherichia coli
  source 1..1917: mol_type = genomic DNA
  CDS 1..1917
atgggtaaaataattggtatcgacctgggtactaccaactcttgtgtagcgattatggatggcaccactcctcgcgtgctggagaacgccgaaggcgatcgcaccacgccttctatcattgcctatacccaggatggtgaaactctagttggtcagccggctaaacgtcaggcagtgacgaacccgcaaaacactctgtttgcgattaaacgcctgattggtcgccgcttccaggacgaagaagtacagcgtgatgtttccatcatgccgttcaaaattattgctgctgataacggcgacgcatgggtcgaagttaaaggccagaaaatggcaccgccgcagatttctgctgaagtgctgaaaaaaatgaagaaaaccgctgaagattacctgggtgaaccggtaactgaagctgttatcaccgtaccggcatactttaacgatgctcagcgtcaggcaaccaaagacgcaggccgtatcgctggtctggaagtaaaacgtatcatcaacgaaccgaccgcagctgcgctggcttacggtctggacaaaggcactggcaaccgtactatcgcggtttatgacctgggtggtggtactttcgatatttctattatcgaaatcgacgaagttgacggcgaaaaaaccttcgaagttctggcaaccaacggtgatacccacctggggggtgaagacttcgacagccgtctgatcaactatctggttgaagaattcaagaaagatcagggcattgacctgcgcaacgatccgctggcaatgcagcgcctgaaagaagcggcagaaaaagcgaaaatcgaactgtcttccgctcagcagaccgacgttaacctgccatacatcactgcagacgcgaccggtccgaaacacatgaacatcaaagtgactcgtgcgaaactggaaagcctggttgaagatctggtaaaccgttccattgagccgctgaaagttgcactgcaggacgctggcctgtccgtatctgatatcgacgacgttatcctcgttggtggtcagactcgtatgccaatggttcagaagaaagttgctgagttctttggtaaagagccgcgtaaagacgttaacccggacgaagctgtagcaatcggtgctgctgttcagggtggtgttctgactggtgacgtaaaagacgtactgctgctggacgttaccccgctgtctctgggtatcgaaaccatgggcggtgtgatgacgacgctgatcgcgaaaaacaccactatcccgaccaagcacagccaggtgttctctaccgctgaagacaaccagtctgcggtaaccatccatgtgctgcagggtgaacgtaaacgtgcggctgataacaaatctctgggtcagttcaacctagatggtatcaacccggcaccgcgcggcatgccgcagatcgaagttaccttcgatatcgatgctgacggtatcctgcacgtttccgcgaaagataaaaacagcggtaaagagcagaagatcaccatcaaggcttcttctggtctgaacgaagatgaaatccagaaaatggtacgcgacgcagaagctaacgccgaagctgaccgtaagtttgaagagctggtacagactcgcaaccagggcgaccatctgctgcacagcacccgtaagcaggttgaagaagcaggcgacaaactgccggctgacgacaaaactgctatcgagtctgcgctgactgcactggaaactgctctgaaaggtgaagacaaagccgctatcgaagcgaaaatgcaggaactggcacaggtttcccagaaactgatggaaatcgcccagcagcaacatgcccagcagcagactgccggtgctgatgcttctgcaaacaacgcgaaagatgacgatgttgtcgacgctgaatttgaagaagtcaaagacaaaaaataa

SEQ ID NO: 6 - protein, 638 aa, Escherichia coli
MGKIIGIDLGTTNSCVAIMDGTTPRVLENAEGDRTTPSIIAYTQDGETLVGQPAKRQAVTNPQNTLFAIKRLIGRRFQDEEVQRDVSIMPFKIIAADNGDAWVEVKGQKMAPPQISAEVLKKMKKTAEDYLGEPVTEAVITVPAYFNDAQRQATKDAGRIAGLEVKRIINEPTAAALAYGLDKGTGNRTIAVYDLGGGTFDISIIEIDEVDGEKTFEVLATNGDTHLGGEDFDSRLINYLVEEFKKDQGIDLRNDPLAMQRLKEAAEKAKIELSSAQQTDVNLPYITADATGPKHMNIKVTRAKLESLVEDLVNRSIEPLKVALQDAGLSVSDIDDVILVGGQTRMPMVQKKVAEFFGKEPRKDVNPDEAVAIGAAVQGGVLTGDVKDVLLLDVTPLSLGIETMGGVMTTLIAKNTTIPTKHSQVFSTAEDNQSAVTIHVLQGERKRAADNKSLGQFNLDGINPAPRGMPQIEVTFDIDADGILHVSAKDKNSGKEQKITIKASSGLNEDEIQKMVRDAEANAEADRKFEELVQTRNQGDHLLHSTRKQVEEAGDKLPADDKTAIESALTALETALKGEDKAAIEAKMQELAQVSQKLMEIAQQQHAQQQTAGADASANNAKDDDVVDAEFEEVKDKK

SEQ ID NO: 7 - DNA, 1914 bp, Pseudomonas aeruginosa
  source 1..1914: mol_type = genomic DNA
  CDS 1..1914
atgggcaaaatcattggcatcgacctgggtaccaccaactcctgcgtggctatcctggagaacggtaacgtcaaggtcatcgagaacgccgagggcgcgcgtaccaccccctcgatcatcgcctacaccaacgatggcgaaaccctggtgggccagccggccaagcgccaggcggtcaccaacccgcagaacaccctgtatgcggtgaagcgcctgatcggccgtcgcttcgaagagaacgtggttcagaaagacatccagatggtgccgtacagcatcgtcaaggccgacaacggcgacgcctgggtggaagtgaagggccagaagatggcgcctccgcagatttccgccgaagtgctgaagaaaatgaagaagaccgccgaagactacctcggcgagccggtcaccgaagcggtgatcaccgttccggcctacttcaacgacagccagcgccaggccaccaaggacgccggccgcatcgccggcctcgacgtcaagcggatcatcaacgagccgaccgcggcggcgctggcctacggcctggacaaggccaagggcgaccacaccgtgatcgtctatgacctgggcggcggtaccttcgacgtgtcggtgatcgagatcgccgaagtcgacggcgagcaccagttcgaagtgctggccaccaacggcgacaccttcctcggcggcgaagacttcgacatccgcctgatcgactacctcgtcgacgagttcaagaaggaaagcggcatcaacctgaagggcgacccgctggccatgcagcgtctgaaggaagcggccgagaaagccaagatcgagctgtcctcgacccagcagaccgacgtcaacctgccgtacgtgactgccgacgcgagcggtccgaagcacctgaacgtcaaggtttcccgcgccaagctggagtccctggtcgaagacctggtgcagcgcaccatcgagccgtgccgcaccgcgctgaaggatgccggcctggatgtttccgatatccatgaagtgatcctggtcggcggccagacccgcatgccgctggtacagaagaccgttgccgagttcttcggcaaggaagcgcgcaaggacgtcaacccggacgaagccgtggctgtcggtgccgccatccagggcgcggtcctggccggcgacgtgaaggacgtgctgctgctcgacgtgaccccgctgaccctcggcatcgagaccctgggcggcgtgatgaccggtctgatcgagaagaacaccaccatcccgaccaagaagtcgcaggtgttctccaccgccgacgacaaccagggcgcggtgaccatccacgtgctgcagggcgagcgcaagcaggccgcgcagaacaagtcgctgggcaagttcgacctggccgacattccgccggctccgcgcggcgtgccgcagatcgaggtgaccttcgatatcgatgccaacggcatcctgcacgtctcggcgaaggacaaggccaccggcaagcagcagtccatcgtgatcaaggcatcctccggcctgtccgaggatgagatccagcagatggtccgcgatgccgaggcgaacgccgaggaggaccgcaagttcgaggaactggctgccgctcgcaaccagggcgacgcgctggtccacgcgacccgcaagatgatcaccgaggcgggcgacaaggccaccgccgaggacaaggcgaccatcgagaaggcgctgggcgagctggaagcggcggtgaagggcgacgacaaggccgagatcgaggccaagatgaacgctctgtcccaggcttccaccccgctggcgcagaagatgtacgccgaacaggcccagcagggcgaagacgctccccagggcgagcaggcgaaagccgctgacgacgtggtggacgccgagttcgaagaggtcaaggacaacaagtaa

SEQ ID NO: 8 - protein, 637 aa, Pseudomonas aeruginosa
MGKIIGIDLGTTNSCVAILENGNVKVIENAEGARTTPSIIAYTNDGETLVGQPAKRQAVTNPQNTLYAVKRLIGRRFEENVVQKDIQMVPYSIVKADNGDAWVEVKGQKMAPPQISAEVLKKMKKTAEDYLGEPVTEAVITVPAYFNDSQRQATKDAGRIAGLDVKRIINEPTAAALAYGLDKAKGDHTVIVYDLGGGTFDVSVIEIAEVDGEHQFEVLATNGDTFLGGEDFDIRLIDYLVDEFKKESGINLKGDPLAMQRLKEAAEKAKIELSSTQQTDVNLPYVTADASGPKHLNVKVSRAKLESLVEDLVQRTIEPCRTALKDAGLDVSDIHEVILVGGQTRMPLVQKTVAEFFGKEARKDVNPDEAVAVGAAIQGAVLAGDVKDVLLLDVTPLTLGIETLGGVMTGLIEKNTTIPTKKSQVFSTADDNQGAVTIHVLQGERKQAAQNKSLGKFDLADIPPAPRGVPQIEVTFDIDANGILHVSAKDKATGKQQSIVIKASSGLSEDEIQQMVRDAEANAEEDRKFEELAAARNQGDALVHATRKMITEAGDKATAEDKATIEKALGELEAAVKGDDKAEIEAKMNALSQASTPLAQKMYAEQAQQGEDAPQGEQAKAADDVVDAEFEEVKDNK

SEQ ID NO: 9 - protein, 7 aa, synthetic construct
  REGION 1..7: note = nuclear localization signal
PKKKRKV

SEQ ID NO: 10 - protein, 5 aa, synthetic construct
  REGION 1..5: note = nuclear localization signal
KKKRK

SEQ ID NO: 11 - protein, 9 aa, synthetic construct
  REGION 1..9: note = nuclear localization signal
PAAKRVKLD

SEQ ID NO: 12 - protein, 7 aa, synthetic construct
  REGION 1..7: note = nuclear localization signal
PQPKKKP

SEQ ID NO: 13 - protein, 6 aa, synthetic construct
  REGION 1..6: note = nuclear localization signal
QRKRQK

SEQ ID NO: 14 - protein, 16 aa, synthetic construct
  REGION 1..16: note = nuclear localization signal
KRPAATKKAGQAKKKK

SEQ ID NO: 15 - protein, 25 aa, synthetic construct
  REGION 1..25: note = nuclear localization signal
MSRRRKANPTKLSENAKKLAKEVEN

SEQ ID NO: 16 - protein, 9 aa, synthetic construct
  REGION 1..9: note = nuclear localization signal
KLKIKRPVK

SEQ ID NO: 17 - DNA, 70 bp, synthetic construct
  misc_feature 1..70: note = polynucleotide for genome editing
  source 1..70: mol_type = other DNA
cggcgtgcagtgcttcagccgctaccccgaccacatgaagcagcacgacttcttcaagtccgccatgccc

SEQ ID NO: 18 - DNA, 731 bp, synthetic construct
  misc_feature 1..731: note = polynucleotide encoding modified GFP with eight nucleotide insertion
  source 1..731: mol_type = other DNA
atggtgagcaagggcgaggagctgttcaccggggtggtgcccatcctggtcgagctggacggcgacgtaaacggccacaagttcagcgtgtccggcgagggcgagggcgatgccacctacggcaagctgaccctgaagttcatctgcaccaccggcaagctgcccgtgccctggcccaccctcgtgaccaccctgacctacggcgtgcagtgcttcagccgctaccccgaccacacggccagctgaagcagcacgacttcttcaagtccgccatgcccgaaggctacgtccaggagcgcaccatcttcttcaaggacgacggcaactacaagacccgcgccgaggtgaagttcgagggcgacaccctggtgaaccgcatcgagctgaagggcatcgacttcaaggaggacggcaacatcctggggcacaagctggagtacaactacaacagccacaacgtctatatcatggccgacaagcagaagaacggcatcaaggtgaacttcaagatccgccacaacatcgaggacggcagcgtgcagctcgccgaccactaccagcagaacacccccatcggcgacggccccgtgctgctgcccgacaaccactacctgagcacccagtccgccctgagcaaagaccccaacgagaagcgcgatcacatggtcctgctggagttcgtgaccgccgccgggatcactctcggcatggacgagctgtacaagtactag

SEQ ID NO: 19 - DNA, 387 bp, synthetic construct
  misc_feature 1..387: note = polynucleotide encoding E.coli Hfq with additional peptides
  source 1..387: mol_type = other DNA
  CDS 1..387
atgggccatcatcatcatcatcatcatcatcatcacagcagcggccatatcgaaggtcgtcatatggctaaggggcaatctttacaagatccgttcctgaacgcactgcgtcgggaacgtgttccagtttctatttatttggtgaatggtattaagctgcaagggcaaatcgagtcttttgatcagttcgtgatcctgttgaaaaacacggtcagccagatggtttacaagcacgcgatttctactgttgtcccgtctcgcccggtttctcatcacagtaacaacgccggtggcggtaccagcagtaactaccatcatggtagcagcgcgcagaatacttccgcgcaacaggacagcgaagaaaccgaaaagaaaaagcgtaagtaa

SEQ ID NO: 20 - protein, 128 aa, synthetic construct
MGHHHHHHHHHHSSGHIEGRHMAKGQSLQDPFLNALRRERVPVSIYLVNGIKLQGQIESFDQFVILLKNTVSQMVYKHAISTVVPSRPVSHHSNNAGGGTSSNYHHGSSAQNTSAQQDSEETEKKKRK

SEQ ID NO: 21 - DNA, 1995 bp, synthetic construct
  misc_feature 1..1995: note = polynucleotide encoding E.coli DnaK with additional peptides
  source 1..1995: mol_type = other DNA
  CDS 1..1995
atgggccatcatcatcatcatcatcatcatcatcacagcagcggccatatcgaaggtcgtcatatgggtaaaataattggtatcgacctgggtactaccaactcttgtgtagcgattatggatggcaccactcctcgcgtgctggagaacgccgaaggcgatcgcaccacgccttctatcattgcctatacccaggatggtgaaactctagttggtcagccggctaaacgtcaggcagtgacgaacccgcaaaacactctgtttgcgattaaacgcctgattggtcgccgcttccaggacgaagaagtacagcgtgatgtttccatcatgccgttcaaaattattgctgctgataacggcgacgcatgggtcgaagttaaaggccagaaaatggcaccgccgcagatttctgctgaagtgctgaaaaaaatgaagaaaaccgctgaagattacctgggtgaaccggtaactgaagctgttatcaccgtaccggcatactttaacgatgctcagcgtcaggcaaccaaagacgcaggccgtatcgctggtctggaagtaaaacgtatcatcaacgaaccgaccgcagctgcgctggcttacggtctggacaaaggcactggcaaccgtactatcgcggtttatgacctgggtggtggtactttcgatatttctattatcgaaatcgacgaagttgacggcgaaaaaaccttcgaagttctggcaaccaacggtgatacccacctggggggtgaagacttcgacagccgtctgatcaactatctggttgaagaattcaagaaagatcagggcattgacctgcgcaacgatccgctggcaatgcagcgcctgaaagaagcggcagaaaaagcgaaaatcgaactgtcttccgctcagcagaccgacgttaacctgccatacatcactgcagacgcgaccggtccgaaacacatgaacatcaaagtgactcgtgcgaaactggaaagcctggttgaagatctggtaaaccgttccattgagccgctgaaagttgcactgcaggacgctggcctgtccgtatctgatatcgacgacgttatcctcgttggtggtcagactcgtatgccaatggttcagaagaaagttgctgagttctttggtaaagagccgcgtaaagacgttaacccggacgaagctgtagcaatcggtgctgctgttcagggtggtgttctgactggtgacgtaaaagacgtactgctgctggacgttaccccgctgtctctgggtatcgaaaccatgggcggtgtgatgacgacgctgatcgcgaaaaacaccactatcccgaccaagcacagccaggtgttctctaccgctgaagacaaccagtctgcggtaaccatccatgtgctgcagggtgaacgtaaacgtgcggctgataacaaatctctgggtcagttcaacctagatggtatcaacccggcaccgcgcggcatgccgcagatcgaagttaccttcgatatcgatgctgacggtatcctgcacgtttccgcgaaagataaaaacagcggtaaagagcagaagatcaccatcaaggcttcttctggtctgaacgaagatgaaatccagaaaatggtacgcgacgcagaagctaacgccgaagctgaccgtaagtttgaagagctggtacagactcgcaaccagggcgaccatctgctgcacagcacccgtaagcaggttgaagaagcaggcgacaaactgccggctgacgacaaaactgctatcgagtctgcgctgactgcactggaaactgctctgaaaggtgaagacaaagccgctatcgaagcgaaaatgcaggaactggcacaggtttcccagaaactgatggaaatcgcccagcagcaacatgcccagcagcagactgccggtgctgatgcttctgcaaacaacgcgaaagatgacgatgttgtcgacgctgaatttgaagaagtcaaagacaaaaaaaagaaaaagcgtaagtaa

SEQ ID NO: 22 - protein, 664 aa, synthetic construct
MGHHHHHHHHHHSSGHIEGRHMGKIIGIDLGTTNSCVAIMDGTTPRVLENAEGDRTTPSIIAYTQDGETLVGQPAKRQAVTNPQNTLFAIKRLIGRRFQDEEVQRDVSIMPFKIIAADNGDAWVEVKGQKMAPPQISAEVLKKMKKTAEDYLGEPVTEAVITVPAYFNDAQRQATKDAGRIAGLEVKRIINEPTAAALAYGLDKGTGNRTIAVYDLGGGTFDISIIEIDEVDGEKTFEVLATNGDTHLGGEDFDSRLINYLVEEFKKDQGIDLRNDPLAMQRLKEAAEKAKIELSSAQQTDVNLPYITADATGPKHMNIKVTRAKLESLVEDLVNRSIEPLKVALQDAGLSVSDIDDVILVGGQTRMPMVQKKVAEFFGKEPRKDVNPDEAVAIGAAVQGGVLTGDVKDVLLLDVTPLSLGIETMGGVMTTLIAKNTTIPTKHSQVFSTAEDNQSAVTIHVLQGERKRAADNKSLGQFNLDGINPAPRGMPQIEVTFDIDADGILHVSAKDKNSGKEQKITIKASSGLNEDEIQKMVRDAEANAEADRKFEELVQTRNQGDHLLHSTRKQVEEAGDKLPADDKTAIESALTALETALKGEDKAAIEAKMQELAQVSQKLMEIAQQQHAQQQTAGADASANNAKDDDVVDAEFEEVKDKKKKKRK

SEQ ID NO: 23 - DNA, 4264 bp, synthetic construct
  misc_feature 1..4264: note = gene cassette for assay plasmid
  source 1..4264: mol_type = other DNA
aagcttccacctgcgtccaggggtggagatcgtcagcgcaacggcggacggcgatctggtggtgcagggcgatctcgatctgtccggctaccgctacgccagcctcaatccgaacacgccgctgaccgaggtctacggttccggcgaggtcggcgcgctggtgctgcgcgccggcggtgacctgaacctctacggcagtatcaacgacggcttcgcgccgccgccggactcgccggacgacaagggctggatcctcaccccgggagtgcagccgttcggtggcgacctggtggttcccggcccgggcgtggtgctcggcgacggtaccgcgttcctcggcggccgcaccctcaactacgacctgccgatcaagggcaccaccctggccgccggcacccgtctggccaccgaggcggtactcgagcagccctataccctggccgccggcagcgtgctggtagcggacatccacgatgccgccggcaccctgctgtacgccgcgggcagcctgctgcgcgacggggtgacgctggaggtcggcagccggctgggtgccggtaccctgctggcggcaccggccagcgtgcaggcgatgacctggcctgcgggcgtgcccttgccgagcatcctgcgcgaggggcccagcagacccaatgtcctgctgctcaatggagagctggccttggcacgtggttctctgatcccttcgcagaccgaggtggtactggctggcgatgcgcctttcatcgagttgcggcccagcgacggtgtccgccagggacgcaactgggcattggccgagatgctgccggccggtagccagtcctggtccatgcgcctggtcgccggtgccgatctcgcggctgccgacaaccgtctggtgcgtccggactcctcggccagcctgaacctggccgatacgcactatcaggcgaagatcgaacagagctcgggagggctggtgttcaccgatcaggctaccgactgggggatcaccccgggaactccggtcgacgagagcaatgaatgacgcgtgttctggcaaatattctgaaatgagctgttgacaattaatcatcggctcgtataatgtgtggaattgtgagcggataacaatttcacacaggaaacagaattccctggaaacgaggaacgccatgaaccgaaacgacctgcgccgcgtcgatctgaacctgctgatcgtgttcgagaccctgatgcacgaacgcagcgtgacccgcgccgcagagaaactgttcctcggccagccggccagccggccatcagcgccgcgctgtcgcgcctgcgcacgctgttcgacgacccgctgttcgtccgtaccggacgcagcatggagcccaccgcgcgagcccaggaaatcttcgcccacctgtcgccggcgctggattccatctccaccgccatgagtcgcgccagcgagttcgatccggcgaccagcaccgcggtgttccgcatcggcctttccgacgacgtcgagttcggcctgttgccgcccctgctccgccgcctgcgcgcggaggcgccggggttcgtcctcgtcgtgcgccgcgccaactatctattgatgccgaacctgctggcctcgggggagatctcggtgggcgtcagctacaccgacgaactgccggccaacgccaagcgcaagaccgtgcgccgcagcaagccgaagatcctccgcgccgactccgcgcccggccagctgaccctcgacgactattgcgcgcgaccgcacgcgctggtgtccttcgccggcgacctcagcggcttcgtcgacgagaagaagatcactggatataccaccgttgatatatcccaatggcatcgtaaagaacattttgaggcatttcagtcagttgctcaatgtacctataaccagaccgttcagctggatattacggcctttttaaagaccgtaaagaaaaataagcacaagttttatccggcctttattcacattcttgcccgcctgatgaatgctcatccggaatttcgtatggcaatgaaagacggtgagctggtgatatgggatagtgttcacccttgttacaccgttttccatgagcaaactgaaacgttttcatcgctctggagtgaataccacgacgatttccggcagtttctacacatatattcgcaagatgtggcgtgttacggtgaaaacctggcctatttccctaaagggtttattgagaatatgtttttcgtctcagccaatccctgggtgagtttcaccagttttgatttaaacgtggccaatatggacaacttcttcgcccccgttttcaccatgggcaaatattatacgcaaggcgacaaggtgctgatgccgctggcgattcaggttcatcatgccgtttgtgatggcttccatgtcggcagaatgcttaatgaattacaacagtactgcgatgagtggcagggcggggcgccagatctgggtaccggtggtggctccggtcatatggtgagcaagggcgaggagctgttcaccggggtggtgcccatcctggtcgagctggacggcgacgtaaacggccacaagttcagcgtgtccggcgagggcgagggcgatgccacctacggcaagctgaccctgaagttcatctgcaccaccggcaagctgcccgtgccctggcccaccctcgtgaccaccctgacctacggcgtgcagtgcttcagccgctaccccgaccacatgaagcagcacgacttcttcaagtccgccatgcccgaaggctacgtccaggagcgcaccatcttcttcaaggacgacggcaactacaagacccgcgccgaggtgaagttcgagggcgacaccctggtgaaccgcatcgagctgaagggcatcgacttcaaggaggacggcaacatcctggggcacaagctggagtacaactacaacagccacaacgtctatatcatggccgacaagcagaagaacggcatcaaggtgaacttcaagatccgccacaacatcgaggacggcagcgtgcagctcgccgaccactaccagcagaacacccccatcggcgacggccccgtgctgctgcccgacaaccactacctgagcacccagtccgccctgagcaaagaccccaacgagaagcgcgatcacatggtcctgctggagttcgtgaccgccgccgggatcactctcggcatggacgagctgtacaagtactagcggccgccgggatccaccggatctaggctagcgtattgtgccgagcctccccgctggacctgggcgcccggcaattacctgggcatgcctgctggtacggcgatcggcgagggcgatctgtggtggtgcagtgtcgatccgtccctgtgtatcgagaatctcggcaaaaccgtggtcacaccgcagaaccagttgttcagtgtgctgcgcaccggcactggcgatcttgacctggccagtgccggtaaccttacgcaatggtcgccgtacggcgtctataccgccggaacgcaggccgccgatgtcgcgacgggattcaatcagcctcgcggtctgttcaatgggtcggtactgggcgccggtggcgcggattacgaagtgctctcaaccagccagtaccaggcctggtatccggaacatggtggcaacctcgatatcgccgttggcggtgatgtggttggcgatcaatgggccgagaaactgacaagtagcgatcccattcgccccttgccccccagcgctgcagtcggcaactggctctggcgccagggcagcgccgatagggaaggagtgccgacggcctggtgggtcaatttcggcagctatgtgcgtggcgcggagggagatgctccctatctggtcggcttcaccggtttcggcactctgggaggcggcaatctcagcatgcgaaccggaggtgatgccggcaatatcgcgccacgcggagatggctcgataccttcgtccggtaaccttaatccgcgcagccagggactggtcttggcggttgccggcactggccggctcacctccgacggcgcgctgcaacttggcggcggcggtgacctgaatgtgagaattggcggggaggtgaacccgagccgggaggcgcgggctacccagacctactcgagttcggggtttgacggtctttacagcggcggcaccattcacgatctgcagggggccctcatcaatctgcgcggttccgcgagcttgtacagtggtgcgctgggaggcatcgatcctcgctacgacactctactgcgggactctaga

SEQ ID NO: 24 - DNA, 22 bp, Pseudomonas aeruginosa
  source 1..22: mol_type = genomic DNA
cggccagccggccagccggcca

SEQ ID NO: 25 - DNA, 84 bp, synthetic construct
  misc_feature 1..84: note = partial sequence of sense strand of polynucleotide encoding modified GFP with eight nucleotide insertion
  source 1..84: mol_type = other DNA
ctacggcgtgcagtgcttcagccgctaccccgaccacacggccagctgaagcagcacgacttcttcaagtccgccatgcccgaa

SEQ ID NO: 26 - DNA, 84 bp, synthetic construct
  misc_feature 1..84: note = partial sequence of antisense strand of polynucleotide encoding modified GFP with eight nucleotide insertion
  source 1..84: mol_type = other DNA
ttcgggcatggcggacttgaagaagtcgtgctgcttcagctggccgtgtggtcggggtagcggctgaagcactgcacgccgtag